European Patent Specification EP 3 858 365 B1, published January 31, 2024. Title: Gold Optimized CAR T-cells. Applicant: Chimera Bioengineering, Inc. The sequence listing filed with the application follows.

SEQUENCE LISTING (32 sequences)

SEQ ID NO: 1 - RNA, 98 nt, Artificial Sequence
  Tetracycline RNA control device
gcgcguccuggauuaaaacauaccagauuucgaucuggagaggugaagaauacgaccaccuaauccagcugaugagucccaaauaggacgaaacgcgc

SEQ ID NO: 2 - RNA, 110 nt, Artificial Sequence
  New tetracycline RNA control device
  misc_feature (16)..(20): n is a, c, g, or u
  misc_feature (70)..(74): n is a, c, g, or u
gcgcguccuggauucnnnnnuaaaacauaccagauuucggucuggagaggugaagaauacgaccaccuannnnnauccagcugaugagucccaaauaggacgaaacgcgc

SEQ ID NO: 3 - RNA, 31 nt, Artificial Sequence
  Aptamer for 6R-folinic acid
acgucgacuuauauugcaugguucgugacgu

SEQ ID NO: 4 - RNA, 37 nt, Artificial Sequence
  Alternative apatamer for 6R-folinic acid
cgaaccggccuuauauugcauggugcguugcggcucg

SEQ ID NO: 5 - RNA, 66 nt, Artificial Sequence
  New aptamer for 6R-folinic acid
gcugucaccggaugcuugguacguuauauucaguccggucugaugaguccgugaggacgaaacagc

SEQ ID NO: 6 - RNA, 76 nt, Artificial Sequence
  Aptamer for 6R-folinic acid
gcugucaccggauggcguugcgugguacguuauauuccggccaucuggucugaugaguccgugaggacgaaacagc

SEQ ID NO: 7 - RNA, 67 nt, Artificial Sequence
  Aptamer for 6R-folinic acid
gcugucaccggauugcgugguacguuauauuccguccggucugaugaguccgugaggacgaaacagc

SEQ ID NO: 8 - RNA, 5 nt, Artificial Sequence
  AU repeat element
auuua

SEQ ID NO: 9 - RNA, 13 nt, Artificial Sequence
  AU rich element
auuuauuuauuua

SEQ ID NO: 10 - RNA, 5 nt, Artificial Sequence
  GU rich repeat element
uuguu

SEQ ID NO: 11 - RNA, 7 nt, Artificial Sequence
  GU rich repeat element
uggggau

SEQ ID NO: 12 - RNA, 5 nt, Artificial Sequence
  U rich repeat element
guuug

SEQ ID NO: 13 - RNA, 7 nt, Artificial Sequence
  GU rich element
uuuguuu

SEQ ID NO: 14 - RNA, 9 nt, Artificial Sequence
  U rich element
  misc_feature (1)..(2): n is a, c, g, or u
  misc_feature (5)..(6): n is a, c, g, or u
nnuunnuuu

SEQ ID NO: 15 - RNA, 7 nt, Artificial Sequence
  U rich element
uuuauuu

SEQ ID NO: 16 - RNA, 7 nt, Artificial Sequence
  U rich element
uuuuuuu

SEQ ID NO: 17 - RNA, 5 nt, Artificial Sequence
  RDE element
uuaga

SEQ ID NO: 18 - RNA, 5 nt, Artificial Sequence
  RDE element
aguuu

SEQ ID NO: 19 - RNA, 9 nt, Artificial Sequence
  RDE element
uuauuuauu

SEQ ID NO: 20 - RNA, 4 nt, Artificial Sequence
  RDE element
uuga

SEQ ID NO: 21 - RNA, 7 nt, Artificial Sequence
  RDE element
uggggau

SEQ ID NO: 22 - RNA, 9 nt, Artificial Sequence
  RDE element
cugcugcug

SEQ ID NO: 23 - RNA, 5 nt, Artificial Sequence
  RDE element
auuga

SEQ ID NO: 24 - protein, 18 aa, Thoseaasigna virus 2A
EGRGSLLTCGDVEENPGP

SEQ ID NO: 25 - protein, 19 aa, Porcine teschovirus-1
ATNFSLLKQAGDVEENPGP

SEQ ID NO: 26 - protein, 20 aa, Equine rhinitis A virus
QCTNYALLKLAGDVESNPGP

SEQ ID NO: 27 - protein, 22 aa, foot and mouth disease virus
VKQTLNFDLLKLAGDVESNPGP

SEQ ID NO: 28 - DNA, 282 bp, Homo sapiens
taattaagtgcttcccacttaaaacatatcaggccttctatttatttaaatatttaaattttatatttattgttgaatgtatggtttgctacctattgtaactattattcttaatcttaaaactataaatatggatcttttatgattctttttgtaagccctaggggctctaaaatggtttcacttatttatcccaaaatatttattattatgttgaatgttaaatatagtatctatgtagattggttagtaaaactatttaataaatttgataaatataaa

SEQ ID NO: 29 - DNA, 282 bp, Homo sapiens
taattaagtgcttcccacttaaaacatatcaggccttctatttatttaaatatttaaattttatatttattgttgaatgtatggtttgctacctattgtaactattattcttaatcttaaaactataaatatggatcttttatgattgaatttgtaagccctaggggctctaaaatggtttcacttatttatcccaaaatatttattattatgttgaatgttaaatatagtatctatgtagattggttagtaaaactatttaataaatttgataaatataaa

SEQ ID NO: 30 - DNA, 585 bp, Homo sapiens
tggttgtcctgcctgcaatatttgaattttaaatctaaatctatttattaatatttaacattatttatatggggaatatatttttagactcatcaatcaaataagtatttataatagcaacttttgtgtaatgaaaatgaatatctattaatatatgtattatttataattcctatatcctgtgactgtctcacttaatcctttgttttctgactaattaggcaaggctatgtgattacaaggctttatctcaggggccaactaggcagccaacctaagcaagatcccatgggttgtgtgtttatttcacttgatgatacaatgaacacttataagtgaagtgatactatccagttactgccggtttgaaaatatgcctgcaatctgagccagtgctttaatggcatgtcagacagaacttgaatgtgtcaggtgaccctgatgaaaacatagcatctcaggagatttcatgcctggtgcttccaaatattgttgacaactgtgactgtacccaaatggaaagtaactcatttgttaaaattatcaatatctaatatatatgaataaagtgtaagttcacaacta

SEQ ID NO: 31 - DNA, 32 bp, Artificial Sequence
  MinP promoter
tagagggtatataatggaagctcgacttccag

SEQ ID NO: 32 - DNA, 131 bp, Artificial Sequence
  NFAT promoter
ggaggaaaaactgtttcatacagaaggcgtggaggaaaaactgtttcatacagaaggcgtggaggaaaaactgtttcatacagaaggcgtagatctagactctagagggtatataatggaagctcgaattc